European Patent Application EP 4 589 018 A2, published July 23, 2025. Title: ENZYME FORMULATIONS AND REACTION MIXTURES FOR NUCLEIC ACID AMPLIFICATION. Applicant: GEN-PROBE INCORPORATED. Application EP. The sequence listing filed with the application follows.

SEQUENCE LISTING (20 sequences)

SEQ ID NO: 1 - DNA, 51 bp, synthetic construct
  misc_feature 1..51: note = Synthetic Oligonucleotide
  source 1..51: mol_type = other DNA
kkkkkkkkkkkkkkkkkktttaaaaaaaaaaaaaaaaaaaaaaaaaaaaaa

SEQ ID NO: 2 - DNA, 14 bp, synthetic construct
  misc_feature 1..14: note = Synthetic Oligonucleotide
  source 1..14: mol_type = other DNA
tttttttttttttt

SEQ ID NO: 3 - DNA, 51 bp, synthetic construct
  misc_feature 1..51: note = Synthetic Oligonucleotide
  source 1..51: mol_type = other DNA
rrrrrrrrrrrrrrrrrrtttaaaaaaaaaaaaaaaaaaaaaaaaaaaaaa

SEQ ID NO: 4 - DNA, 20 bp, synthetic construct
  misc_feature 1..20: note = Synthetic Oligonucleotide
  source 1..20: mol_type = other DNA
gatgtggtggttttggacat

SEQ ID NO: 5 - DNA, 24 bp, synthetic construct
  misc_feature 1..24: note = Synthetic Oligonucleotide
  source 1..24: mol_type = other DNA
cttcttagaaaacttacccttagg

SEQ ID NO: 6 - DNA, 26 bp, synthetic construct
  misc_feature 1..26: note = Synthetic Oligonucleotide
  source 1..26: mol_type = other DNA
agttgaagatgcttatgaccaggtgc

SEQ ID NO: 7 - RNA, 552 nt, synthetic construct
  misc_feature 1..552: note = Synthetic Oligonucleotide
  source 1..552: mol_type = other RNA
gggcgaattgggtaccgggccccccctcgaggtcgacggtatcgataagcttatctgtctgtgagaccgatgctgtgaatcagcaatctgttcacaagtggcacacactagaccaaaagcagcttctgtggtcactgttcccatcctgttgtatatgaggcccatgcaactggcaagtgcaccagttgaatagcttagtgacacctccttggccccatggaacgttatttctcttttgagcttcttgtatagtttaactgctctatccatgttgttcgggtccccattcccatttagggcattttggacaaagcgtctacgctgcagtcctcgctcactgggcacggtgagcgtgaacacaaatcctaaaattcccttagtcagaggtgacaagattggtcttgtctttagccattccatgagagcctcaagatctgtgttctttcctgcaaagacactttccagtctctgcgcgatctcggctttgagggggcctgacgggatgatagaaagaacgtacgtttcgacctcggttagaagactcatgcggcc

SEQ ID NO: 8 - DNA, 22 bp, synthetic construct
  misc_feature 1..22: note = Synthetic Oligonucleotide
  source 1..22: mol_type = other DNA
cttctaaccgaggtcgaaacgt

SEQ ID NO: 9 - DNA, 19 bp, synthetic construct
  misc_feature 1..19: note = Synthetic Oligonucleotide
  source 1..19: mol_type = other DNA
cccttagtcagaggtgaca

SEQ ID NO: 10 - DNA, 20 bp, synthetic construct
  misc_feature 1..20: note = Synthetic Oligonucleotide
  source 1..20: mol_type = other DNA
ataacgttccatggggccaa

SEQ ID NO: 11 - DNA, 20 bp, synthetic construct
  misc_feature 1..20: note = Synthetic Oligonucleotide
  source 1..20: mol_type = other DNA
cccatyctgttgtatatgag

SEQ ID NO: 12 - DNA, 26 bp, synthetic construct
  misc_feature 1..26: note = Synthetic Oligonucleotide
  source 1..26: mol_type = other DNA
tcaggccccctcaaagccgagatcgc

SEQ ID NO: 13 - DNA, 26 bp, synthetic construct
  source 1..26: mol_type = other DNA
  misc_feature 1..5: note = DNA
  misc_feature 6: note = RNA
  misc_feature 7..26: note = DNA
agccattccatgagagcctcaagatc

SEQ ID NO: 14 - DNA, 23 bp, synthetic construct
  source 1..23: mol_type = other DNA
  misc_feature 1..19: note = DNA
  misc_feature 20: note = RNA
  misc_feature 21..23: note = DNA
ctggtgcacttgccagttgtatg

SEQ ID NO: 15 - DNA, 23 bp, synthetic construct
  misc_feature 1..23: note = Synthetic Oligonucleotide
  source 1..23: mol_type = other DNA
ccctacttgagccaargaactaa

SEQ ID NO: 16 - DNA, 23 bp, synthetic construct
  misc_feature 1..23: note = Synthetic Oligonucleotide
  source 1..23: mol_type = other DNA
ggcctaacwcctcaaacatatgc

SEQ ID NO: 17 - DNA, 26 bp, synthetic construct
  misc_feature 1..26: note = Synthetic Oligonucleotide
  source 1..26: mol_type = other DNA
ttaaagcagcaaacccagcaatagcc

SEQ ID NO: 18 - DNA, 20 bp, synthetic construct
  misc_feature 1..20: note = Synthetic Oligonucleotide
  source 1..20: mol_type = other DNA
ttaggagacgccctcaatcg

SEQ ID NO: 19 - DNA, 20 bp, synthetic construct
  misc_feature 1..20: note = Synthetic Oligonucleotide
  source 1..20: mol_type = other DNA
tggccagaaatacaccaaca

SEQ ID NO: 20 - DNA, 22 bp, synthetic construct
  misc_feature 1..22: note = Synthetic Oligonucleotide
  source 1..22: mol_type = other DNA
ccgtgtattcccccgcactaaa